European Patent Application EP 4 803 546 A1, published September 9, 2026. Title: 结合HLA-A24/PRAME复合体的多种抗体及其用途. Applicant: 北京智仁美博生物科技有限公司. The sequence listing filed with the application follows.

SEQUENCE LISTING (98 sequences)

SEQ ID NO: 1 - protein, 5 aa, Llama
IYVMG

SEQ ID NO: 2 - protein, 16 aa, Llama
VITGSGNTNYADSVKG

SEQ ID NO: 3 - protein, 16 aa, Llama
GRPSRYYRDSGTWADF

SEQ ID NO: 4 - protein, 124 aa, Llama
QVQLVESGGGLVQAGGSLRLSCAASGASLDIYVMGWYRQATGKERDLVAVITGSGNTNYADSVKGRFTISRDDAKNTLYLQMSSLKPEDTAVYYCAGGRPSRYYRDSGTWADFWGQGTQVTVSS

SEQ ID NO: 5 - protein, 124 aa, synthetic construct
EVQLVESGGGLVKPGGSLRLSCAASGASLDIYVMGWYRQAPGKGLELVAVITGSGNTNYADSVKGRFTISRDDSKNTLYLQMNSLKTEDTAVYYCAGGRPSRYYRDSGTWADFWGQGTTVTVSS

SEQ ID NO: 6 - protein, 5 aa, synthetic construct
GYTMN

SEQ ID NO: 7 - protein, 17 aa, synthetic construct
LINPYKGVSTYNQKFKD

SEQ ID NO: 8 - protein, 13 aa, synthetic construct
SGYYGDSDWYFDV

SEQ ID NO: 9 - protein, 11 aa, synthetic construct
RASQDIRNYLN

SEQ ID NO: 10 - protein, 7 aa, synthetic construct
YTSRLES

SEQ ID NO: 11 - protein, 9 aa, synthetic construct
QQGNTLPWT

SEQ ID NO: 12 - protein, 122 aa, synthetic construct [sequence omitted]

SEQ ID NO: 13 - protein, 107 aa, synthetic construct [sequence omitted]

SEQ ID NO: 14 - protein, 263 aa, synthetic construct
QVQLVESGGGLVQAGGSLRLSCAASGASLDIYVMGWYRQATGKERDLVAVITGSGNTNYADSVKGRFTISRDDAKNTLYLQMSSLKPEDTAVYYCAGGRPSRYYRDSGTWADFWGQGTQVTVSSGGGGSGGGGSGGGGSQVQLVESGGGLVQAGGSLRLSCAASGASLDIYVMGWYRQATGKERDLVAVITGSGNTNYADSVKGRFTISRDDAKNTLYLQMSSLKPEDTAVYYCAGGRPSRYYRDSGTWADFWGQGTQVTVSS

SEQ ID NO: 15 - protein, 263 aa, synthetic construct
EVQLVESGGGLVKPGGSLRLSCAASGASLDIYVMGWYRQAPGKGLELVAVITGSGNTNYADSVKGRFTISRDDSKNTLYLQMNSLKTEDTAVYYCAGGRPSRYYRDSGTWADFWGQGTTVTVSSGGGGSGGGGSGGGGSEVQLVESGGGLVKPGGSLRLSCAASGASLDIYVMGWYRQAPGKGLELVAVITGSGNTNYADSVKGRFTISRDDSKNTLYLQMNSLKTEDTAVYYCAGGRPSRYYRDSGTWADFWGQGTTVTVSS

SEQ ID NO: 16 - protein, 253 aa, synthetic construct
DIQMTQSPSSLSASVGDRVTITCRASQDIRNYLNWYQQKPGKAPKLLIYYTSRLESGVPSRFSGSGSGTDYTLTISSLQPEDFATYYCQQGNTLPWTFGQGTKVEIKGGGGSGGGGSGGGGSGGGGSGGGSEVQLVESGGGLVQPGGSLRLSCAASGYSFTGYTMNWVRQAPGKGLEWVALINPYKGVSTYNQKFKDRFTISVDKSKNTAYLQMNSLRAEDTAVYYCARSGYYGDSDWYFDVWGQGTLVTVSS

SEQ ID NO: 17 - protein, 105 aa, homo sapiens
QDGNEEMGGITQTPYKVSISGTTVILTCPQYPGSEILWQHNDKNIGGDEDDKNIGSDEDHLSLKEFSELEQSGYYVCYPRGSKPEDANFYLYLRARVCENCMEMD

SEQ ID NO: 18 - protein, 84 aa, homo sapiens [sequence omitted]

SEQ ID NO: 19 - protein, 9 aa, homo sapiens
LYVDSLFFL

SEQ ID NO: 20 - protein, 418 aa, synthetic construct
LYVDSLFFLGCGGSGGGGSGGGGSIQRTPKIQVYSRHPAENGKSNFLNCYVSGFHPSDIEVDLLKNGERIEKVEHSDLSFSKDWSFYLLYYTEFTPTEKDEYACRVNHVTLSQPKIVKWDRDMGGGGSGGGGSGGGGSGGGGSGSHSMRYFSTSVSRPGRGEPRFIAVGYVDDTQFVRFDSDAASQRMEPRAPWIEQEGPEYWDEETGKVKAHSQTDRENLRIALRCYNQSEAGSHTLQMMFGCDVGSDGRFLRGYHQYAYDGKDYIALKEDLRSWTAADMAAQITKRKWEAAHVAEQQRAYLEGTCVDGLRRYLENGKETLQRTDPPKTHMTHHPISDHEATLRCWALGFYPAEITLTWQRDGEDQTQDTELVETRPAGDGTFQKWAAVVVPSGEEQRYTCHVQHEGLPKPLTLRWE

SEQ ID NO: 21 - protein, 6 aa, synthetic construct
HHHHHH

SEQ ID NO: 22 - protein, 234 aa, mus musculus
ASPRGPTIKPCPPCKCPAPNLLGGPSVFIFPPKIKDVLMISLSPIVTCVVVDVSEDDPDVQISWFVNNVEVHTAQTQTHREDYNSTLRVVSALPIQHQDWMSGKEFKCKVNNKDLPAPIERTISKPKGSVRAPQVYVLPPPEEEMTKKQVTLTCMVTDFMPEDIYVEWTNNGKTELNYKNTEPVLDSDGSYFMYSKLRVEKKNWVERNSYSCSVVHEGLHNHHTTKSFSRTPGK

SEQ ID NO: 23 - protein, 330 aa, homo sapiens
ASTKGPSVFPLAPSSKSTSGGTAALGCLVKDYFPEPVTVSWNSGALTSGVHTFPAVLQSSGLYSLSSVVTVPSSSLGTQTYICNVNHKPSNTKVDKRVEPKSCDKTHTCPPCPAPELLGGPSVFLFPPKPKDTLMISRTPEVTCVVVDVSHEDPEVKFNWYVDGVEVHNAKTKPREEQYNSTYRVVSVLTVLHQDWLNGKEYKCKVSNKALPAPIEKTISKAKGQPREPQVYTLPPSREEMTKNQVSLTCLVKGFYPSDIAVEWESNGQPENNYKTTPPVLDSDGSFFLYSKLTVDKSRWQQGNVFSCSVMHEALHNHYTQKSLSLSPGK

SEQ ID NO: 24 - protein, 330 aa, synthetic construct
ASTKGPSVFPLAPSSKSTSGGTAALGCLVKDYFPEPVTVSWNSGALTSGVHTFPAVLQSSGLYSLSSVVTVPSSSLGTQTYICNVNHKPSNTKVDKRVEPKSCDKTHTCPPCPAPELLGGPSVFLFPPKPKDTLMISRTPEVTCVVVDVSHEDPEVKFNWYVDGVEVHNAKTKPREEQYNSTYRVVSVLTVLHQDWLNGKEYKCKVSNKALPAPIEKTISKAKGQPREPQVCTLPPSREEMTKNQVSLSCAVKGFYPSDIAVEWESNGQPENNYKTTPPVLDSDGSFFLVSKLTVDKSRWQQGNVFSCSVMHEALHNHYTQKSLSLSPGK

SEQ ID NO: 25 - protein, 330 aa, synthetic construct
ASTKGPSVFPLAPSSKSTSGGTAALGCLVKDYFPEPVTVSWNSGALTSGVHTFPAVLQSSGLYSLSSVVTVPSSSLGTQTYICNVNHKPSNTKVDKRVEPKSCDKTHTCPPCPAPELLGGPSVFLFPPKPKDTLMISRTPEVTCVVVDVSHEDPEVKFNWYVDGVEVHNAKTKPREEQYNSTYRVVSVLTVLHQDWLNGKEYKCKVSNKALPAPIEKTISKAKGQPREPQVYTLPPCREEMTKNQVSLWCLVKGFYPSDIAVEWESNGQPENNYKTTPPVLDSDGSFFLYSKLTVDKSRWQQGNVFSCSVMHEALHNHYTQKSLSLSPGK

SEQ ID NO: 26 - protein, 330 aa, synthetic construct
ASTKGPSVFPLAPSSKSTSGGTAALGCLVKDYFPEPVTVSWNSGALTSGVHTFPAVLQSSGLYSLSSVVTVPSSSLGTQTYICNVNHKPSNTKVDKRVEPKSCDKTHTCPPCPAPEFEGGPSVFLFPPKPKDTLMISRTPEVTCVVVDVSHEDPEVKFNWYVDGVEVHNAKTKPREEQYNSTYRVVSVLTVLHQDWLNGKEYKCKVSNKALPASIEKTISKAKGQPREPQVCTLPPSREEMTKNQVSLSCAVKGFYPSDIAVEWESNGQPENNYKTTPPVLDSDGSFFLVSKLTVDKSRWQQGNVFSCSVMHEALHNHYTQKSLSLSPGK

SEQ ID NO: 27 - protein, 330 aa, synthetic construct
ASTKGPSVFPLAPSSKSTSGGTAALGCLVKDYFPEPVTVSWNSGALTSGVHTFPAVLQSSGLYSLSSVVTVPSSSLGTQTYICNVNHKPSNTKVDKRVEPKSCDKTHTCPPCPAPEFEGGPSVFLFPPKPKDTLMISRTPEVTCVVVDVSHEDPEVKFNWYVDGVEVHNAKTKPREEQYNSTYRVVSVLTVLHQDWLNGKEYKCKVSNKALPASIEKTISKAKGQPREPQVYTLPPCREEMTKNQVSLWCLVKGFYPSDIAVEWESNGQPENNYKTTPPVLDSDGSFFLYSKLTVDKSRWQQGNVFSCSVMHEALHNHYTQKSLSLSPGK

SEQ ID NO: 28 - protein, 327 aa, synthetic construct
ASTKGPSVFPLAPSSKSTSEGTAALGCLVKDYFPEPVTVSWNSGALTSGVHTFPAVLQSSGLYSLSSVVTVPSSSLGTQTYICNVDHKPSNTKVDKTVERKSCVECPPCPAPEFEGGPSVFLFPPKPKDTLMISRTPEVTCVVVDVSQEDPEVQFNWYVDGVEVHNAKTKPREEQYNSTYRVVSVLTVLHQDWLNGKEYKCKVSNKALPASIEKTISKAKGQPREPQVCTLPPSQEEMTKNQVSLSCAVKGFYPSDIAVEWESNGQPENNYKTTPPVLDSDGSFFLVSKLTVDKSRWQEGNVFSCSVMHEALHNHYTQKSLSLSPGK

SEQ ID NO: 29 - protein, 327 aa, synthetic construct
ASTKGPSVFPLAPSSKSTSGGTAALGCLVKDYFPEPVTVSWNSGALTSGVHTFPAVLQSSGLYSLSSVVTVPSSSLGTQTYICNVNHKPSNTKVDKRVERKSCVECPPCPAPEFEGGPSVFLFPPKPKDTLMISRTPEVTCVVVDVSHEDPEVKFNWYVDGVEVHNAKTKPREEQYNSTYRVVSVLTVLHQDWLNGKEYKCKVSNKALPASIEKTISKAKGQPREPQVYTLPPCREEMTKNQVSLWCLVKGFYPSDIAVEWESNGQPENNYKTTPPVLDSDGSFFLYSKLTVDKSRWQQGNVFSCSVMHEALHNHYTQKSLSLSPGK

SEQ ID NO: 30 - protein, 106 aa, homo sapiens
GQPKAAPSVTLFPPSSEELQANKATLVCLISDFYPGAVTVAWKADSSPVKAGVETTTPSKQSNNKYAASSYLSLTPEQWKSHRSYSCQVTHEGSTVEKTVAPTECS

SEQ ID NO: 31 - protein, 107 aa, homo sapiens [sequence omitted]

SEQ ID NO: 32 - protein, 234 aa, homo sapiens
ASEPKSSDKTHTCPPCPAPELLGGPSVFLFPPKPKDTLMISRTPEVTCVVVDVSHEDPEVKFNWYVDGVEVHNAKTKPREEQYNSTYRVVSVLTVLHQDWLNGKEYKCKVSNKALPAPIEKTISKAKGQPREPQVYTLPPSRDELTKNQVSLTCLVKGFYPSDIAVEWESNGQPENNYKTTPPVLDSDGSFFLYSKLTVDKSRWQQGNVFSCSVMHEALHNHYTQKSLSLSPGK

SEQ ID NO: 33 - protein, 231 aa, synthetic construct
ASERKSSVECPPCPAPEFEGGPSVFLFPPKPKDTLMISRTPEVTCVVVDVSQEDPEVQFNWYVDGVEVHNAKTKPREEQYNSTYRVVSVLTVLHQDWLNGKEYKCKVSNKALPASIEKTISKAKGQPREPQVCTLPPSQEEMTKNQVSLSCAVKGFYPSDIAVEWESNGQPENNYKTTPPVLDSDGSFFLVSKLTVDKSRWQEGNVFSCSVMHEALHNHYTQKSLSLSPGK

SEQ ID NO: 34 - protein, 231 aa, synthetic construct
ASERKSSVECPPCPAPEFEGGPSVFLFPPKPKDTLMISRTPEVTCVVVDVSHEDPEVKFNWYVDGVEVHNAKTKPREEQYNSTYRVVSVLTVLHQDWLNGKEYKCKVSNKALPASIEKTISKAKGQPREPQVYTLPPCREEMTKNQVSLWCLVKGFYPSDIAVEWESNGQPENNYKTTPPVLDSDGSFFLYSKLTVDKSRWQQGNVFSCSVMHEALHNHYTQKSLSLSPGK

SEQ ID NO: 35 - protein, 494 aa, synthetic construct
QVQLVESGGGLVQAGGSLRLSCAASGASLDIYVMGWYRQATGKERDLVAVITGSGNTNYADSVKGRFTISRDDAKNTLYLQMSSLKPEDTAVYYCAGGRPSRYYRDSGTWADFWGQGTQVTVSSGGGGSGGGGSGGGGSQVQLVESGGGLVQAGGSLRLSCAASGASLDIYVMGWYRQATGKERDLVAVITGSGNTNYADSVKGRFTISRDDAKNTLYLQMSSLKPEDTAVYYCAGGRPSRYYRDSGTWADFWGQGTQVTVSSASERKSSVECPPCPAPEFEGGPSVFLFPPKPKDTLMISRTPEVTCVVVDVSQEDPEVQFNWYVDGVEVHNAKTKPREEQYNSTYRVVSVLTVLHQDWLNGKEYKCKVSNKALPASIEKTISKAKGQPREPQVCTLPPSQEEMTKNQVSLSCAVKGFYPSDIAVEWESNGQPENNYKTTPPVLDSDGSFFLVSKLTVDKSRWQEGNVFSCSVMHEALHNHYTQKSLSLSPGK

SEQ ID NO: 36 - protein, 494 aa, synthetic construct
EVQLVESGGGLVKPGGSLRLSCAASGASLDIYVMGWYRQAPGKGLELVAVITGSGNTNYADSVKGRFTISRDDSKNTLYLQMNSLKTEDTAVYYCAGGRPSRYYRDSGTWADFWGQGTTVTVSSGGGGSGGGGSGGGGSEVQLVESGGGLVKPGGSLRLSCAASGASLDIYVMGWYRQAPGKGLELVAVITGSGNTNYADSVKGRFTISRDDSKNTLYLQMNSLKTEDTAVYYCAGGRPSRYYRDSGTWADFWGQGTTVTVSSASERKSSVECPPCPAPEFEGGPSVFLFPPKPKDTLMISRTPEVTCVVVDVSQEDPEVQFNWYVDGVEVHNAKTKPREEQYNSTYRVVSVLTVLHQDWLNGKEYKCKVSNKALPASIEKTISKAKGQPREPQVCTLPPSQEEMTKNQVSLSCAVKGFYPSDIAVEWESNGQPENNYKTTPPVLDSDGSFFLVSKLTVDKSRWQEGNVFSCSVMHEALHNHYTQKSLSLSPGK

SEQ ID NO: 37 - protein, 484 aa, synthetic construct
DIQMTQSPSSLSASVGDRVTITCRASQDIRNYLNWYQQKPGKAPKLLIYYTSRLESGVPSRFSGSGSGTDYTLTISSLQPEDFATYYCQQGNTLPWTFGQGTKVEIKGGGGSGGGGSGGGGSGGGGSGGGSEVQLVESGGGLVQPGGSLRLSCAASGYSFTGYTMNWVRQAPGKGLEWVALINPYKGVSTYNQKFKDRFTISVDKSKNTAYLQMNSLRAEDTAVYYCARSGYYGDSDWYFDVWGQGTLVTVSSASERKSSVECPPCPAPEFEGGPSVFLFPPKPKDTLMISRTPEVTCVVVDVSHEDPEVKFNWYVDGVEVHNAKTKPREEQYNSTYRVVSVLTVLHQDWLNGKEYKCKVSNKALPASIEKTISKAKGQPREPQVYTLPPCREEMTKNQVSLWCLVKGFYPSDIAVEWESNGQPENNYKTTPPVLDSDGSFFLYSKLTVDKSRWQQGNVFSCSVMHEALHNHYTQKSLSLSPGK

SEQ ID NO: 38 - protein, 509 aa, homo sapiens
MERRRLWGSIQSRYISMSVWTSPRRLVELAGQSLLKDEALAIAALELLPRELFPPLFMAAFDGRHSQTLKAMVQAWPFTCLPLGVLMKGQHLHLETFKAVLDGLDVLLAQEVRPRRWKLQVLDLRKNSHQDFWTVWSGNRASLYSFPEPEAAQPMTKKRKVDGLSTEAEQPFIPVEVLVDLFLKEGACDELFSYLIEKVKRKKNVLRLCCKKLKIFAMPMQDIKMILKMVQLDSIEDLEVTCTWKLPTLAKFSPYLGQMINLRRLLLSHIHASSYISPEKEEQYIAQFTSQFLSLQCLQALYVDSLFFLRGRLDQLLRHVMNPLETLSITNCRLSEGDVMHLSQSPSVSQLSVLSLSGVMLTDVSPEPLQALLERASATLQDLVFDECGITDDQLLALLPSLSHCSQLTTLSFYGNSISISALQSLLQHLIGLSNLTHVLYPVPLESYEDIHGTLHLERLAYLHARLRELLCELGRPSMVWLSANPCPHCGDRTFYDPEPILCPCFMPN

SEQ ID NO: 39 - protein, 333 aa, homo sapiens
MESSGNPESTTFFYYDLQSQPCENQAWVFATLATTVLYCLVFLLSLVGNSLVLWVLVKYESLESLTNIFILNLCLSDLVFACLLPVWISPYHWGWVLGDFLCKLLNMIFSISLYSSIFFLTIMTIHRYLSVVSPLSTLRVPTLRCRVLVTMAVWVASILSSILDTIFHKVLSSGCDYSELTWYLTSVYQHNLFFLLSLGIILFCYVEILRTLFRSRSKRRHRTVKLIFAIVVAYFLSWGPYNFTLFLQTLFRTQIIRSCEAKQQLEYALLICRNLAFSHCCFNPVLYVFVGVKFRTHLKHVLRQFWFCRLQAPSPASIPHSPGAFAYEGASFY

SEQ ID NO: 40 - protein, 621 aa, homo sapiens
MANVPWAEVCEKFQAALALSRVELHKNPEKEPYKSKYSARALLEEVKALLGPAPEDEDERPEAEDGPGAGDHALGLPAEVVEPEGPVAQRAVRLAVIEFHLGVNHIDTEELSAGEEHLVKCLRLLRRYRLSHDCISLCIQAQNNLGILWSEREEIETAQAYLESSEALYNQYMKEVGSPPLDPTERFLPEEEKLTEQERSKRFEKVYTHNLYYLAQVYQHLEMFEKAAHYCHSTLKRQLEHNAYHPIEWAINAATLSQFYINKLCFMEARHCLSAANVIFGQTGKISATEDTPEAEGEVPELYHQRKGEIARCWIKYCLTLMQNAQLSMQDNIGELDLDKQSELRALRKKELDEEESIRKKAVQFGTGELCDAISAVEEKVSYLRPLDFEEARELFLLGQHYVFEAKEFFQIDGYVTDHIEVVQDHSALFKVLAFFETDMERRCKMHKRRIAMLEPLTVDLNPQYYLLVNRQIQFEIAHAYYDMMDLKVAIADRLRDPDSHIVKKINNLNKSALKYYQLFLDSLRDPNKVFPEHIGEDVLRPAMLAKFRVARLYGKIITADPKKELENLATSLEHYKFIVDYCEKHPEAAQEIEVELELSKEMVSLLPTKMERFRTKMALT

SEQ ID NO: 41 - protein, 476 aa, homo sapiens
MVGAMWKVIVSLVLLMPGPCDGLFRSLYRSVSMPPKGDSGQPLFLTPYIEAGKIQKGRELSLVGPFPGLNMKSYAGFLTVNKTYNSNLFFWFFPAQIQPEDAPVVLWLQGGPGGSSMFGLFVEHGPYVVTSNMTLRDRDFPWTTTLSMLYIDNPVGTGFSFTDDTHGYAVNEDDVARDLYSALIQFFQIFPEYKNNDFYVTGESYAGKYVPAIAHLIHSLNPVREVKINLNGIAIGDGYSDPESIIGGYAEFLYQIGLLDEKQKKYFQKQCHECIEHIRKQNWFEAFEILDKLLDGDLTSDPSYFQNVTGCSNYYNFLRCTEPEDQLYYVKFLSLPEVRQAIHVGNQTFNDGTIVEKYLREDTVQSVKPWLTEIMNNYKVLIYNGQLDIIVAAALTERSLMGMDWKGSQEYKKAEKKVWKIFKSDSEVAGYIRQVGDFHQVIIRGGGHILPYDQPLRAFDMINRFIYGKGWDPYVG

SEQ ID NO: 42 - protein, 1074 aa, homo sapiens
MSLKNEPRVNTSALQKIAADMSNIIENLDTRELHFEGEEVDYDVSPSDPKIQEVYIPFSAIYNTQGFKEPNIQTYLSGCPIKAQVLEVERFTSTTRVPSINLYTIELTHGEFKWQVKRKFKHFQEFHRELLKYKAFIRIPIPTRRHTFRRQNVREEPREMPSLPRSSENMIREEQFLGRRKQLEDYLTKILKMPMYRNYHATTEFLDISQLSFIHDLGPKGIEGMIMKRSGGHRIPGLNCCGQGRACYRWSKRWLIVKDSFLLYMKPDSGAIAFVLLVDKEFKIKVGKKETETKYGIRIDNLSRTLILKCNSYRHARWWGGAIEEFIQKHGTNFLKDHRFGSYAAIQENALAKWYVNAKGYFEDVANAMEEANEEIFITDWWLSPEIFLKRPVVEGNRWRLDCILKRKAQQGVRIFIMLYKEVELALGINSEYTKRTLMRLHPNIKVMRHPDHVSSTVYLWAHHEKLVIIDQSVAFVGGIDLAYGRWDDNEHRLTDVGSVKRVTSGPSLGSLPPAAMESMESLRLKDKNEPVQNLPIQKSIDDVDSKLKGIGKPRKFSKFSLYKQLHRHHLHDADSISSIDSTSSYFNHYRSHHNLIHGLKPHFKLFHPSSESEQGLTRPHADTGSIRSLQTGVGELHGETRFWHGKDYCNFVFKDWVQLDKPFADFIDRYSTPRMPWHDIASAVHGKAARDVARHFIQRWNFTKIMKSKYRSLSYPFLLPKSQTTAHELRYQVPGSVHANVQLLRSAADWSAGIKYHEESIHAAYVHVIENSRHYIYIENQFFISCADDKVVFNKIGDAIAQRILKAHRENQKYRVYVVIPLLPGFEGDISTGGGNALQAIMHFNYRTMCRGENSILGQLKAELGNQWINYISFCGLRTHAELEGNLVTELIYVHSKLLIADDNTVIIGSANINDRSMLGKRDSEMAVIVQDTETVPSVMDGKEYQAGRFARGLRLQCFRVVLGYLDDPSEDIQDPVSDKFFKEVWVSTAARNATIYDKVFRCLPNDEVHNLIQLRDFINKPVLAKEDPIRAEEELKKIRGFLVQFPFYFLSEESLLPSVGTKEAIVPMEVWT

SEQ ID NO: 43 - protein, 339 aa, homo sapiens
HSMRYFSTSVSRPGRGEPRFIAVGYVDDTQFVRFDSDAASQRMEPRAPWIEQEGPEYWDEETGKVKAHSQTDRENLRIALRYYNQSEAGSHTLQMMFGCDVGSDGRFLRGYHQYAYDGKDYIALKEDLRSWTAADMAAQITKRKWEAAHVAEQQRAYLEGTCVDGLRRYLENGKETLQRTDPPKTHMTHHPISDHEATLRCWALGFYPAEITLTWQRDGEDQTQDTELVETRPAGDGTFQKWAAVVVPSGEEQRYTCHVQHEGLPKPLTLRWEPSSQPTIPIVGIIAGLVLFGAVITGAVVAAVMWRRKSSDRKGGSYSQAASSDSAQGSDVSLTACKV

SEQ ID NO: 44 - protein, 9 aa, homo sapiens
SYVRSLPFF

SEQ ID NO: 45 - protein, 9 aa, homo sapiens
TYTDRVFFL

SEQ ID NO: 46 - protein, 9 aa, homo sapiens
TYVDWHFLL

SEQ ID NO: 47 - protein, 9 aa, homo sapiens
LYPKTLFLL

SEQ ID NO: 48 - protein, 9 aa, homo sapiens
LYPSTLFLL

SEQ ID NO: 49 - protein, 9 aa, homo sapiens
IYKDSSTFL

SEQ ID NO: 50 - protein, 9 aa, homo sapiens
SYVASFFLL

SEQ ID NO: 51 - protein, 9 aa, homo sapiens
VYQHNLFFL

SEQ ID NO: 52 - protein, 9 aa, homo sapiens
YYGPSLFLL

SEQ ID NO: 53 - protein, 9 aa, homo sapiens
LMTDVLVFL

SEQ ID NO: 54 - protein, 9 aa, homo sapiens
VYTHNLYYL

SEQ ID NO: 55 - protein, 9 aa, homo sapiens
TYNSNLFFW

SEQ ID NO: 56 - protein, 9 aa, homo sapiens
AYDDKIYYF

SEQ ID NO: 57 - protein, 9 aa, homo sapiens
AYMPHTFFI

SEQ ID NO: 58 - protein, 9 aa, homo sapiens
AYELTQYYF

SEQ ID NO: 59 - protein, 9 aa, homo sapiens
IYIENQFFI

SEQ ID NO: 60 - protein, 9 aa, homo sapiens
NYQRLFDFF

SEQ ID NO: 61 - protein, 9 aa, homo sapiens
RYILEPFFI

SEQ ID NO: 62 - protein, 9 aa, homo sapiens
KYPLNLYLL

SEQ ID NO: 63 - protein, 9 aa, homo sapiens
GYISSAFLF

SEQ ID NO: 64 - protein, 9 aa, homo sapiens
TYLLSVYRL

SEQ ID NO: 65 - protein, 9 aa, homo sapiens
VYSNSIYEL

SEQ ID NO: 66 - protein, 9 aa, homo sapiens
PYISNIYLI

SEQ ID NO: 67 - protein, 9 aa, homo sapiens
KTKSMFFFL

SEQ ID NO: 68 - protein, 9 aa, homo sapiens
DMKTKYFFF

SEQ ID NO: 69 - protein, 9 aa, homo sapiens
NYIDKVRFL

SEQ ID NO: 70 - protein, 9 aa, homo sapiens
IYDPNLAFL

SEQ ID NO: 71 - protein, 9 aa, homo sapiens
IYEPNFIFF

SEQ ID NO: 72 - protein, 9 aa, homo sapiens
LYQDKFPFF

SEQ ID NO: 73 - protein, 9 aa, homo sapiens
QYASAFHFL

SEQ ID NO: 74 - protein, 9 aa, homo sapiens
KYLEMIYSM

SEQ ID NO: 75 - protein, 9 aa, homo sapiens
KYDPNVYSI

SEQ ID NO: 76 - protein, 9 aa, homo sapiens
EYLRQIFRL

SEQ ID NO: 77 - protein, 9 aa, homo sapiens
SYSPQAFKF

SEQ ID NO: 78 - protein, 9 aa, homo sapiens
VFLGQAFTI

SEQ ID NO: 79 - protein, 9 aa, homo sapiens
EYAVMLYTW

SEQ ID NO: 80 - protein, 9 aa, homo sapiens
YYLPQLYEL

SEQ ID NO: 81 - protein, 9 aa, homo sapiens
RYLVTLYGF

SEQ ID NO: 82 - protein, 9 aa, homo sapiens
TYIKSPPFF

SEQ ID NO: 83 - protein, 9 aa, homo sapiens
KYGIVQEFF

SEQ ID NO: 84 - protein, 9 aa, homo sapiens
SYADAFQFL

SEQ ID NO: 85 - protein, 9 aa, homo sapiens
VYQLRFQFL

SEQ ID NO: 86 - protein, 9 aa, homo sapiens
SYIPSTVFF

SEQ ID NO: 87 - protein, 9 aa, homo sapiens
SYLDSVHFF

SEQ ID NO: 88 - protein, 9 aa, homo sapiens
IYDFIGEFM

SEQ ID NO: 89 - protein, 9 aa, homo sapiens
YYDLVKAFM

SEQ ID NO: 90 - protein, 9 aa, homo sapiens
IYKPVTDFF

SEQ ID NO: 91 - protein, 9 aa, homo sapiens
VYENVSHFL

SEQ ID NO: 92 - protein, 9 aa, homo sapiens
HYILHNSFF

SEQ ID NO: 93 - protein, 9 aa, homo sapiens
AYEIIDQFF

SEQ ID NO: 94 - protein, 15 aa, synthetic construct
GGGGSGGGGSGGGGS

SEQ ID NO: 95 - DNA, 22 bp, synthetic construct
  source 1..22: mol_type = other DNA
tccttccccgtcagccagtcct

SEQ ID NO: 96 - protein, 115 aa, synthetic construct
EVQLLESGGGLVQPGGSLRLSCAASGFTFSSYAMSWVRQAPGKGLEWVSAISGSGGSTYYADSVKGRFTISRDNSKNTLYLQMNSLRAEDTAVYYCAKGSGFDYWGQGTLVTVSS

SEQ ID NO: 97 - protein, 108 aa, synthetic construct
EIVLTQSPGTLSLSPGERATLSCRASQSVSSSYLAWYQQKPGQAPRLLIYGASSRATGIPDRFSGSGSGTDFTLTISRLEPEDFAVYYCQQYGSSPLTFGQGTKVEIK

SEQ ID NO: 98 - protein, 9 aa, synthetic construct
TYGPVFMCL